European Patent Application EP 4 663 747 A1, published December 17, 2025. Title: TRANSFORMED MICROORGANISM AND POLYHYDROXYALKANOATE PRODUCTION METHOD. Applicant: KANEKA CORPORATION. Application JP. The sequence listing filed with the application follows.

SEQUENCE LISTING (28 sequences)

SEQ ID NO: 1 - protein, 862 aa, Cupriavidus necator
MRLDKLTTRFQEALADAQSLALANDNQYIDPQHVLRALLSQDDGAAKALLSRAGVNVQGLQTALDAAIKRLPQVQGTSEVQIGRDLVNLLNATEKEAIKRGDQFIASELFLLAVADDKGEAGRIARESGLNRKSLESAIQAVRGGESVNSAEAEGQREALKKYTIDLTERARIGKLDPVIGRDDEIRRAIQILQRRTKNNPVLIGEPGVGKTAIVEGLAQRIVNGEVPESLKNKRVLVLDMAGLLAGAKYRGEFEERLKAVLNDVAKDEGQTIVFIDEIHTMVGAGKAEGAIDAGNMLKPALARGELHCIGATTLDEYRKYIEKDAALERRFQKVLVDEPTVEATIAILRGLQEKYELHHGVEITDPAIVAAAELSHRYITDRFLPDKAIDLIDEAAARIKMEIDSKPEAMDKLERRTIQLKIEREAVKKETDEASLKRLDLIEQEIARLEKEYADLDEIWKAEKGAAQGTAALKEEIEKVKLEITKLQREGKLDKVAELQYGKLPGLEGKLKAATDAEASEQKQPNKLLRTQVGAEEIAEVVSRATGIPVSKMMQGEREKLLKMEDRLHARVVGQDEAVRLVSDAIRRSRAGLADENRPYGSFLFLGPTGVGKTELCKALAEFMFDSQEHLIRIDMSEFMEKHSVSRLIGAPPGYVGYEEGGYLTEAVRRKPYSVVLLDEVEKAHPDVFNVLLQVLDDGRLTDGQGRTVDFKNTVIVMTSNLGSQIIQAMTGEPQEAIKGAVWQEVRTHFRPEFLNRIDEVVVFHALDQQHIESIARIQLQRLQARLARMDMTLEVSETALEKIASAGYDPVFGARPLKRAIQQQIENPVARAILEGKFTAKDVVPVDYVDGEFTFGRKLD

SEQ ID NO: 2 - protein, 857 aa, Escherichia coli
MRLDRLTNKFQLALADAQSLALGHDNQFIEPLHLMSALLNQEGGSVSPLLTSAGINAGQLRTDINQALNRLPQVEGTGGDVQPSQDLVRVLNLCDKLAQKRGDNFISSELFVLAALESRGTLADILKAAGATTANITQAIEQMRGGESVNDQGAEDQRQALKKYTIDLTERAEQGKLDPVIGRDEEIRRTIQVLQRRTKNNPVLIGEPGVGKTAIVEGLAQRIINGEVPEGLKGRRVLALDMGALVAGAKYRGEFEERLKGVLNDLAKQEGNVILFIDELHTMVGAGKADGAMDAGNMLKPALARGELHCVGATTLDEYRQYIEKDAALERRFQKVFVAEPSVEDTIAILRGLKERYELHHHVQITDPAIVAAATLSHRYIADRQLPDKAIDLIDEAASSIRMQIDSKPEELDRLDRRIIQLKLEQQALMKESDEASKKRLDMLNEELSDKERQYSELEEEWKAEKASLSGTQTIKAELEQAKIAIEQARRVGDLARMSELQYGKIPELEKQLEAATQLEGKTMRLLRNKVTDAEIAEVLARWTGIPVSRMMESEREKLLRMEQELHHRVIGQNEAVDAVSNAIRRSRAGLADPNRPIGSFLFLGPTGVGKTELCKALANFMFDSDEAMVRIDMSEFMEKHSVSRLVGAPPGYVGYEEGGYLTEAVRRRPYSVILLDEVEKAHPDVFNILLQVLDDGRLTDGQGRTVDFRNTVVIMTSNLGSDLIQERFGELDYAHMKELVLGVVSHNFRPEFINRIDEVVVFHPLGEQHIASIAQIQLKRLYKRLEERGYEIHISDEALKLLSENGYDPVYGARPLKRAIQQQIENPLAQQILSGELVPGKVIRLEVNEDRIVAVQ

SEQ ID NO: 3 - protein, 908 aa, Saccharomyces cerevisiae
MNDQTQFTERALTILTLAQKLASDHQHPQLQPIHILAAFIETPEDGSVPYLQNLIEKGRYDYDLFKKVVNRNLVRIPQQQPAPAEITPSYALGKVLQDAAKIQKQQKDSFIAQDHILFALFNDSSIQQIFKEAQVDIEAIKQQALELRGNTRIDSRGADTNTPLEYLSKYAIDMTEQARQGKLDPVIGREEEIRSTIRVLARRIKSNPCLIGEPGIGKTAIIEGVAQRIIDDDVPTILQGAKLFSLDLAALTAGAKYKGDFEERFKGVLKEIEESKTLIVLFIDEIHMLMGNGKDDAANILKPALSRGQLKVIGATTNNEYRSIVEKDGAFERRFQKIEVAEPSVRQTVAILRGLQPKYEIHHGVRILDSALVTAAQLAKRYLPYRRLPDSALDLVDISCAGVAVARDSKPEELDSKERQLQLIQVEIKALERDEDADSTTKDRLKLARQKEASLQEELEPLRQRYNEEKHGHEELTQAKKKLDELENKALDAERRYDTATAADLRYFAIPDIKKQIEKLEDQVAEEERRAGANSMIQNVVDSDTISETAARLTGIPVKKLSESENEKLIHMERDLSSEVVGQMDAIKAVSNAVRLSRSGLANPRQPASFLFLGLSGSGKTELAKKVAGFLFNDEDMMIRVDCSELSEKYAVSKLLGTTAGYVGYDEGGFLTNQLQYKPYSVLLFDEVEKAHPDVLTVMLQMLDDGRITSGQGKTIDCSNCIVIMTSNLGAEFINSQQGSKIQESTKNLVMGAVRQHFRPEFLNRISSIVIFNKLSRKAIHKIVDIRLKEIEERFEQNDKHYKLNLTQEAKDFLAKYGYSDDMGARPLNRLIQNEILNKLALRILKNEIKDKETVNVVLKKGKSRDENVPEEAEECLEVLPNHEATIGADTLGDDDNEDSMEIDDDLD

SEQ ID NO: 4 - protein, 392 aa, cupriavidus sp. strain S-6
MTDVVIVSAARTAVGKFGGSLAKVPAPELGAIVIKAALERAGVKPEQVSEVIMGQVLTAGSGQNPARQAAIKAGLPHMVPAMTINKVCGSGLKAVMLAANAIASGDAEIVVAGGQENMSAAPHVLPGSRDGFRMGDAKLIDTMIVDGLWDVYNQYHMGITAENVAKEYGISREAQDEFAVSSQNKAEAAQKAGRFDEEIVPVMIPQRKGEPVAFATDEFVRHGATLESIAGLKPAFDKAGTVTAANASGINDGAAAVVVMSAAKARELGLTPLATIRAFANAGVDPKVMGMGPVPASQRCLSRAGWSVQDLDLMEINEAFAAQALAVHKQMGWDTDKVNVNGGAIAIGHPIGASGCRILVTLLHEMKRRDAKKGLASLCIGGGMGVALAVER

SEQ ID NO: 5 - protein, 392 aa, Caldimonas manganoxidans
MSDIVIVSAARTAVGKFGGTLARTPAAELGAVVIAEALRRAGIAGEQVSEVIMGQVLQAGCGQNPARQAVIKAGLPHAVPAMTINKVCGSGLKAVMLAAQAIRDGDAEVVVAGGQENMSQAPHVLLGSREGQRMGDWKMIDSMITDGLWDVYNQYHMGITAENVAKKYGISREEQDALALASQQKAAAAQDAGRFRDEIVAVNIPQKKGDPIVFDTDEFINRKTSAEALAGLRPAFDKAGSVTAGNASGINDGAAAVVVMSAKKADQLGLKPLARIASYASAGLDPAYMGMGPVPAARKALERAGWKAADLDLLEINEAFAAQACAVHKEMGWDTSKVNVNGGAIAIGHPIGASGCRILVTLLYEMQRRRARKGLASLCIGGGMGVALTVER

SEQ ID NO: 6 - protein, 392 aa, Schlegelella thermodepolymerans
MSDIVIVSAARTAVGKFGGTLAKTPAAELGATVIKEVLRRAGLSGEQVSEVIMGQVLQAGCGQNPARQAVIKAGLPEGVPAMTINKVCGSGLKAVMLAAQAIRDGDADIVVAGGQENMSLAPHVLLGSREGQRMGDWKMVDSMITDGLWDVYNQYHMGITAENVAKKYGISREEQDALALASQQKAAAAQDAGRFKDEIVPVVIPQRKGDPVVFDTDEFINRKTSAEALAGLRPAFDKAGTVTAGNASGINDGAAAVVVMSAKRAEQLGLKPLARIASYASAGLDPAYMGMGPVPAARKALDRAGWKPADLDLLEINEAFAAQACAVHKEMGWDTSKVNVNGGAIAIGHPIGASGCRILVTLLHEMQRRDARKGIASLCIGGGMGVALTVER

SEQ ID NO: 7 - protein, 246 aa, cupriavidus sp. strain S-6
MTQRIAYVTGGMGGIGTAICQRLAKDGFRVIAGCGPNSPRRERWLEQQKALGFDFIASEGNVADWDSTKAAFDKVKAEVGEVDVLINNAGITRDVVFRKMTRADWDAVIDTNLTSLFNVTKQVIDGMADRGWGRIINISSVNGQKGQFGQTNYSTAKAGLHGFTMALAQEVATKGVTVNTVSPGYIATDMVKAIRQDVLDKIVGTIPVKRLGQPEEIASICAWLASEESGFATGADFSLNGGLHMG

SEQ ID NO: 8 - protein, 245 aa, Caldimonas manganoxidans
MSQKVAYVTGGMGGIGTAICQRLARSGFKVIAGCGPSRDYQKWLDQQKELGYTFYASVGNVADWDSTVQAFAKAKAEHGPIDVLVNNAGITRDRMFLKMTPEDWHAVIDTNLNSMFNVTKQVVPDMVERGWGRIIQISSVNGEKGQAGQTNYSAAKAGMHGFTMALAQELASKGVTVNTVSPGYISTDMVRAIKPEVLEKIIATIPVKRLGTPEEIASIVAWIASEDSGFATGADFSINGGLHMG

SEQ ID NO: 9 - protein, 245 aa, Schlegelella thermodepolymerans
MAQKVAYVTGGMGGIGTAICQRLARDGFKVIAGCGPNRDYQKWLDQQKELGYTFYASVGNVADWDSTVAAFAKAKAEHGPIDVLVNNAGITRDRMFLKMTPEDWHAVINTNLNSMFNVTKQVVPDMVERGWGRIIQISSVNGEKGQAGQTNYSAAKAGMHGFTMALAQELASKGVTVNTVSPGYIGTDMVRAIKPEILEKIIATIPVRRLGTPEEIASIVSWVASEESGFATGADFSINGGLHMG

SEQ ID NO: 10 - DNA, 29 bp, Escherichia coli
  source 1..29: mol_type = other DNA
ttgacaattaatcatccggctcgtataat

SEQ ID NO: 11 - DNA, 30 bp, Escherichia coli
  source 1..30: mol_type = other DNA
tttacactttatgcttccggctcgtataat

SEQ ID NO: 12 - DNA, 30 bp, Escherichia coli
  source 1..30: mol_type = other DNA
ttgacaattaatcatcgaactagttaacta

SEQ ID NO: 13 - DNA, 30 bp, Escherichia coli
  source 1..30: mol_type = other DNA
tttacactttatgcttccggctcgtatgtt

SEQ ID NO: 14 - DNA, 29 bp, Escherichia coli
  source 1..29: mol_type = other DNA
tttacacttatgcttccggctcgtatgtt

SEQ ID NO: 15 - DNA, 31 bp, Escherichia coli
  source 1..31: mol_type = other DNA
tttacacctttatgcttccggctcgtatgtt

SEQ ID NO: 16 - DNA, 30 bp, Cupriavidus necator
  source 1..30: mol_type = other DNA
ttgacagcgcgtgcgttgcaaggcaacaat

SEQ ID NO: 17 - DNA, 17 bp, Cupriavidus necator
  source 1..17: mol_type = other DNA
agagagacaatcaaatc

SEQ ID NO: 18 - DNA, 2627 bp, Cupriavidus necator
  source 1..2627: mol_type = other DNA
gaaacaattgcagagagacaatcaaatcatgcgtcttgacaagctgaccacccggttccaggaagcactggctgatgcgcaaagcctggcactgggcaacgacaaccaatacatcgaaccgcagcacctgctgcgcgcactgctggcgcaggacgacggcgccgccaaggcgctgctggcgcgcgccggcgtcaacgtgcagggcctgcagacggcgctcgacgccgccatcaagcgcctgccgcaagtgcagggcaccagcgaggtccagatcggccgcgacctggtcaacctgctcaacgccaccgagaaggaagccatcaagcgcggcgaccagttcatcgccagcgagctgttcctgctggccgtcgccgacgacaagggcgacgccggccgcatcgcgcgtgaaaacggcctgaaccgcaagtcgctcgagtcggccatccaggccgtgcgcggcggcgattcggtcaacagcgccgaggccgagggccagcgcgaggccctcaagaagtacaccatcgacctgaccgagcgcgcccgcatcggcaagctcgatcccgtgatcggccgtgacgacgagatccgccgcgccatccagatcctgcagcgccgcaccaagaacaacccggtgctgatcggcgagccgggcgtgggcaagaccgccatcgtggaaggcctggcgcagcgcatcgtcaacggcgaagtgccggagagcctgaagaacaagcgcgtgctggtgctggacatggccggcctgctggccggcgccaagtaccgcggcgagttcgaggagcgcctgaaagcggtgctgaacgacgtcgccaaggacgagggccagaccatcgtcttcatcgacgagatccacaccatggtcggcgccggcaaggccgagggcgcgatcgacgcgggcaacatgctcaagccggcgctcgcgcgcggcgagctgcactgcatcggcgcgaccacgctggacgagtaccgcaagtacatcgagaaggacgccgcgctggagcgccgcttccagaaggtgctggtcgatgagccgagcgttgaagccaccattgccatcctgcgcgggctgcaggaaaagtatgagctgcaccacggcgtggaaatcaccgacccggccatcgtcgccgcggcggagctgtcgcatcgctatatcaccgaccgcttccttcccgacaaggcgatcgacctgatcgacgaggcggccgcgcgcatcaagatggaaatcgattccaagccggagtcgatggacaagctcgagcgccgcaccatccagctgaagatcgagcgcgaggcggtcaagaaagagaccgatgaggcgtcgatgaagcgcctggagctgatcgagcaggaaatcgcgcgcctggagaaggagtacgccgacctggacgagatctggaaagccgagaagggcgccgcgcagggcacggccgcgctcaaggaagagatcgagaaggtcaagctggagatcgccaagctgcagcgcgaaggcaagctggacaaggtggccgagctgcaatacggcaagctgccgggcctggaaggcaagctcaaggcggcgaccgatgccgaggccagcgagcagaagcagcccaacaagctgctgcgcacccaggtgggcgccgaggaaatcgccgaagtggtaagccgcgccaccggcatcccggtatcgaagatgatgcagggcgagcgcgagaagctgctcaagatggaagaccggctgcatgggcgcgtggtcggccaggacgaagccgtgcggctggtgtccgatgccatccgccgttcgcgtgccgggcttgcggacgagaaccggccctatggctcgttcctgttcctgggcccgaccggcgtcggcaagaccgagttgtgcaaggccctggccgagttcatgttcgattcggaagagcacctgatccgcatcgacatgagcgaattcatggagaagcacagcgtcagccgcctgatcggcgcgccgcccggatacgtgggctacgaggaaggcggctacctgaccgaggccgtgcgccgcaagccgtacagcgtggtgctgctggatgaagtcgagaaggcccacccggacgtcttcaacgtgctgctgcaggtgctggacgacggccgcctgaccgatggccagggccgcaccgtggacttcaagaacacggtgatcgtgatgacgtccaacctgggttcgcagatcatccagtcgatgaccggcgagccgcaggaagcgatcaagggtgcggtctggcaggaagtgcgcacgcatttccggccggagttcctgaaccggatcgatgaagtggtggtgttccacgcgctcgaccagaagcatatcgagtcgatcgcacgcatccagctgcaacgcctgcaggcccgcctggcccgcatggacatgacgctggaggtgagcgagacggcgctggagaagatcgccagcgcaggctacgacccggtgtttggcgcgcgtccgctcaagcgggcgatccagcagcagatcgagaacccggtggcccgggcgatcctggaaggcaagttcgccgccaaggatgtggtgccggtggattatgtcgacggggagttcacgttcgggcggaagctggactaaactagtcctg

SEQ ID NO: 19 - protein, 594 aa, Aeromonas sp.
MSQPSYGPLFEALAHYNDKLLAMAKAQTERTAQALLQTNLDDLGQVLEQGSQQPWQLIQAQMNWWQDQLKLMQHTLLKSAGQPSEPVITPERSDRRFKAEAWSEQPIYDYLKQSYLLTARHLLASVDALEGVPQKSRERLRFFTRQYVSAMAPSNFLATNPELLKLTLESGGQNLVRGLALLAEDLERSADQLNIRLTDESAFELGRDLALTPGRVVQRTELYELIQYSPTTETVGKTPVLIVPPFINKYYIMDMRPQNSLVAWLVAQGQTVFMISWRNPGVAQAQIDLDDYVVDGVIAALDGVEAATGEREVHGIGYCIGGTALSLAMGWLAARRQKQRVRTATLFTTLLDFSQPGELGIFIHEPIIAALEAQNEAKGIMDGRQLAVSFSLLRENSLYWNYYIDSYLKGQSPVAFDLLHWNSDSTNVAGKTHNSLLRRLYLENQLVKGELKIRNTRIDLGKVKTPVLLVSAVDDHIALWQGTWQGMKLFGGEQRFLLAESGHIAGIINPPAANKYGFWHNGAEAESPESWLAGATHQGGSWWPEMMGFIQNRDEGSEPVPARVPEEGLAPAPGHYVKVRLNPVFACPTEEDAA

SEQ ID NO: 20 - DNA, 2644 bp, Escherichia coli
  source 1..2644: mol_type = other DNA
gaaacaattgcagagagacaatcaaatcatgcgtctggatcgtcttactaataaattccagcttgctcttgccgatgcccaatcacttgcactcgggcacgacaaccaatttatcgaaccacttcatttaatgagcgccctgctgaatcaggaagggggttcggttagtcctttattaacatccgctggcataaatgctggccagttgcgcacagatatcaatcaggcattaaatcgtttaccgcaggttgaaggtactggtggtgatgtccagccatcacaggatctggtgcgcgttcttaatctttgcgacaagctggcgcaaaaacgtggtgataactttatctcgtcagaactgttcgttctggcggcacttgagtctcgcggcacgctggccgacatcctgaaagcagcaggggcgaccaccgccaacattactcaagcgattgaacaaatgcgtggaggtgaaagcgtgaacgatcaaggtgctgaagaccaacgtcaggctttgaaaaaatataccatcgaccttaccgaacgagccgaacagggcaaactcgatccggtgattggtcgtgatgaagaaattcgccgtaccattcaggtgctgcaacgtcgtactaaaaataacccggtactgattggtgaacccggcgtcggtaaaactgccatcgttgaaggtctggcgcagcgtattatcaacggcgaagtgccggaagggttgaaaggccgccgggtactggcgctggatatgggcgcgctggtggctggggcgaaatatcgcggtgagtttgaagaacgtttaaaaggcgtgcttaacgatcttgccaaacaggaaggcaacgtcatcctatttatcgacgaattacataccatggtcggcgcgggtaaagccgatggcgcaatggacgccggaaacatgctgaaaccggcgctggcgcgtggtgaattgcactgcgtaggtgccacgacgcttgacgaatatcgccagtacattgaaaaagatgctgcgctggaacgtcgtttccagaaagtgtttgttgccgagccttctgttgaagataccattgcgattctgcgtggcctgaaagaacgttacgaattgcaccaccatgtgcaaattactgacccggcaattgttgcagcggcgacgttgtctcatcgctacattgctgaccgtcagctgccggataaagccatcgacctgatcgatgaagcagcatccagcattcgtatgcagattgactcaaaaccagaagaactcgaccgactcgatcgtcgtatcatccagctcaaactggaacaacaggcgttaatgaaagagtctgatgaagccagtaaaaaacgtctggatatgctcaacgaagaactgagcgacaaagaacgtcagtactccgagttagaagaagagtggaaagcagagaaggcatcgctttctggtacgcagaccattaaagcggaactggaacaggcgaaaatcgctattgaacaggctcgccgtgtgggggacctggcgcggatgtctgaactgcaatacggcaaaatcccggaactggaaaagcaactggaagccgcaacgcagctcgaaggcaaaactatgcgtctgttgcgtaataaagtgaccgacgccgaaattgctgaagtgctggcgcgttggacggggattccggtttctcgcatgatggaaagcgagcgcgaaaaactgctgcgtatggagcaagaactgcaccatcgcgtaattggtcagaacgaagcggttgatgcggtatctaacgctattcgtcgtagccgtgcggggctggcggatccaaatcgcccgattggttcattcctgttcctcggcccaactggtgtggggaaaacagagctttgtaaggcgctggcgaactttatgtttgatagcgacgaggcgatggtccgtatcgatatgtccgagtttatggagaaacactcggtgtctcgtttggttggtgcgcctccgggatatgtcggttatgaagaaggtggctacctgaccgaagcggtgcgtcgtcgtccgtattccgtcatcctgctggatgaagtggaaaaagcgcatccggatgtcttcaacattctgttgcaggtactggatgatgggcgtctgactgacgggcaagggagaacggtcgacttccgtaatacggtcgtcattatgacctctaacctcggttccgatctgattcaggaacgcttcggtgaactggattatgcgcacatgaaagagctggtgctcggtgtggtaagccataacttccgtccggaattcattaaccgtatcgatgaagtggtggtcttccatccgctgggtgaacagcacattgcctcgattgcgcagattcagttgaaacgtctgtacaaacgtctggaagaacgtggttatgaaatccacatttctgacgaggcgctgaaactgctgagcgagaacggttacgatccggtctatggtgcacgtcctctgaaacgtgcaattcagcagcagatcgaaaacccgctggcacagcaaatactgtctggtgaattggttccgggtaaagtgattcgcctggaagttaatgaagaccggattgtcgccgtccagtaacctgccggcctggttcaaccagtcggcagccgactagtggat

SEQ ID NO: 21 - protein, 96 aa, Cupriavidus necator
MNLRPLHDRVIVKRLDNETKTASGIVIPDNAAEKPDQGEVLAIGPGKKDDKGNNIALDVKVGDRVLFGKYAGQAVKVEGQELLVMREEDIMAVVNK

SEQ ID NO: 22 - DNA, 2051 bp, Cupriavidus necator
  source 1..2051: mol_type = other DNA
gaaacaattgcagagagacaatcaaatcatgaatctgcgtcctttgcacgaccgcgtgatcgtgaagcgtctggacaacgaaaccaagaccgcgtccggtatcgtgattcccgacaacgctgccgagaagcccgatcaaggcgaagtgctggcaatcggtcctggcaagaaggatgacaagggcaacaacatcgccctcgacgtcaaggtcggtgaccgcgtgctgttcggcaagtacgccggccaggccgtgaaggtggaaggccaggaactgctggtcatgcgcgaagaagacatcatggccgtggtgaacaagtaattcaccaactgaccgccaccccgtacagatttcaggagattcaagaatggcagctaaagacgtagtgttcggcgacgccgcacgtgccaagatggtcgaaggcgtgaacatcctcgccaacgcagtcaaggtgaccctgggcccgaagggccgcaacgtggtgctggagcgcagcttcggcggcccgaccgtgaccaaggacggcgtgtccgtggccaaggaaatcgagctgaaggacaagctgcagaacatgggcgcccagatggtcaaggaagtggcttccaagaccagcgacaacgccggtgacggtaccaccaccgctaccgtgctggcccagtcgatcgtgcgcgaaggcatgaagttcgttgccgccggcatgaacccgatggacctgaagcgcggcatcgacaaggctgttgccgccgccgtggaagagctgaagaaggtcagcaagcccaccaccaccagcaaggaaatcgcccaggttggcgcgatctcggccaacagcgacacctccatcggtgagcgcatcgccgaagccatggacaaggtcggcaaggaaggcgtgatcacggttgaagacggcaagtcgctggccgacgagctggaagtcgtggaaggcatgcagttcgaccgcggctatctgtcgccgtacttcatcaacaacccggaaaagcaggttgtccagctggacaacccgttcgtgctgctgttcgacaagaagatcagcaacatccgcgacctgctgccggtgctggagcaagtggccaaggccggccgcccgctgctgatcgtcgctgaagacgtcgagggcgaagccctggcgaccctagtggtcaacaacatccgtggcatcctgaagaccgccgccgtcaaggccccgggcttcggcgaccgccgcaaggccatgctggaagacatcgccatcctgaccggcggcaccgtcatcgctgaagaaatcggcctgacgctggaaaaggctggcctgaacgacctgggccaggccaagcgcatcgagatcggcaaggaaaacaccatcatcatcgacggcgccggcgacgcagctgcgatcgaaggccgcgtcaagcaaatccgcgcccagatcgaagaagcgacctcggactacgaccgtgagaagctgcaagagcgcgtggccaagctggccggcggtgttgccgtgatcaaggttggcgctgccaccgaagtcgaaatgaaggaaaagaaggcccgcgtggaagacgccctgcacgccacccgcgctgcggtggaagaaggcatcgtccccggcggtggtgtggccctgctgcgtgcccgcgctgcgatctcggcactgaccggcgaaaacgccgaccagaacgccggtatcaagatcgtgctgcgcgccatggaagagccgctgcgccagatcgtgctgaacgccggtgaagaagcttcggtggtcgttgccaaggttatcgaaggcaagggcaactacggctacaacgccgcttcgggcgagtacggcgacctggtggaaatgggcgtgctggacccgaccaaggtcacccgcaccgcactgcagaacgccgcttcggtggcttcgctgatgctgaccaccgactgcgcagttgccgaatcgccgaaggaagaatcggctccggcaatgccgggcggcatgggcggcatgggcggcatggaaggcatgatgtaacctgccggcctggttcaaccagtcggcagccgactagtggat

SEQ ID NO: 23 - DNA, 2051 bp, synthetic construct; identical to SEQ ID NO: 22
  source 1..2051: mol_type = other DNA

SEQ ID NO: 24 - protein, 638 aa, Escherichia coli
MGKIIGIDLGTTNSCVAIMDGTTPRVLENAEGDRTTPSIIAYTQDGETLVGQPAKRQAVTNPQNTLFAIKRLIGRRFQDEEVQRDVSIMPFKIIAADNGDAWVEVKGQKMAPPQISAEVLKKMKKTAEDYLGEPVTEAVITVPAYFNDAQRQATKDAGRIAGLEVKRIINEPTAAALAYGLDKGTGNRTIAVYDLGGGTFDISIIEIDEVDGEKTFEVLATNGDTHLGGEDFDSRLINYLVEEFKKDQGIDLRNDPLAMQRLKEAAEKAKIELSSAQQTDVNLPYITADATGPKHMNIKVTRAKLESLVEDLVNRSIEPLKVALQDAGLSVSDIDDVILVGGQTRMPMVQKKVAEFFGKEPRKDVNPDEAVAIGAAVQGGVLTGDVKDVLLLDVTPLSLGIETMGGVMTTLIAKNTTIPTKHSQVFSTSEDNQSAVTIHVLQGERKRAADNKSLGQFNLDGINPAPRGMPQIEVTFDIDADGILHVSAKDKNSGKEQKITIKASSGLNEDEIQKMVRDAEANAEADRKFEELVQTRNQGDHLLHSTRKQVEEAGDKLPADDKTAIESALTALETALKGEDKAAIEAKMQELAQVSQKLMEIAQQQHAQQQTAGADASANNAKDDDVVDAEFEEVKDKK

SEQ ID NO: 25 - protein, 292 aa, Escherichia coli
MHQGGVNSLALALTAAFCGANQHNHGLLVSWALQGEGMACAPWYVRQRLRRASGRCGSCAALVFSFAPSIRLRGLKNVITITYRVKKREKTCKYDLKVVLLFHRKGNGPSHNSPAGQEIKKMNIQEALNVFGLSGELTEKDIKAAYRKAALKYHPDRNPLGAELMKAVNAAFDVLMANIDKINQFQSTDEHARYNYGDDLEKVLNVLSGLSGLVFEVIGNWVWISGETITHKETLKEIGCKWAAKKKQWFYRPDEHKSYWNREEHTIEEIRAKYGTTGQRRATGWQRVETRA

SEQ ID NO: 26 - DNA, 3206 bp, synthetic construct
  source 1..3206: mol_type = other DNA
gaaacaattgcagagagacaatcaaatcatgggtaaaataattggtatcgacctgggtactaccaactcttgtgtagcgattatggatggcaccactcctcgcgtgctggagaacgccgaaggcgatcgcaccacgccttctatcattgcctatacccaggatggtgaaactctagttggtcagccggctaaacgtcaggcagtgacgaacccgcaaaacactctgtttgcgattaaacgcctgattggtcgccgcttccaggacgaagaagtacagcgtgatgtttccatcatgccgttcaaaattattgctgctgataacggcgacgcatgggtcgaagttaaaggccagaaaatggcaccgccgcagatttctgctgaagtgctgaaaaaaatgaagaaaaccgctgaagattacctgggtgaaccggtaactgaagctgttatcaccgtaccggcatactttaacgatgctcagcgtcaggcaaccaaagacgcaggccgtatcgctggtctggaagtaaaacgtatcatcaacgaaccgaccgcagctgcgctggcttacggtctggacaaaggcactggcaaccgtactatcgcggtttatgacctgggtggtggtactttcgatatttctattatcgaaatcgacgaagttgacggcgaaaaaaccttcgaagttctggcaaccaacggtgatacccacctggggggtgaagacttcgacagccgtctgatcaactatctggttgaagaattcaagaaagatcagggcattgacctgcgcaacgatccgctggcaatgcagcgcctgaaagaagcggcagaaaaagcgaaaatcgaactgtcttccgctcagcagaccgacgttaacctgccatacatcactgcagacgcgaccggtccgaaacacatgaacatcaaagtgactcgtgcgaaactggaaagcctggttgaagatctggtaaaccgttccattgagccgctgaaagttgcactgcaggacgctggcctgtccgtatctgatatcgacgacgttatcctcgttggtggtcagactcgtatgccaatggttcagaagaaagttgctgagttctttggtaaagagccgcgtaaagacgttaacccggacgaagctgtagcaatcggtgctgctgttcagggtggtgttctgactggtgacgtaaaagacgtactgctgctggacgttaccccgctgtctctgggtatcgaaaccatgggcggtgtgatgacgacgctgatcgcgaaaaacaccactatcccgaccaagcacagccaggtgttctctaccgctgaagacaaccagtctgcggtaaccatccatgtgctgcagggtgaacgtaaacgtgcggctgataacaaatctctgggtcagttcaacctagatggtatcaacccggcaccgcgcggcatgccgcagatcgaagttaccttcgatatcgatgctgacggtatcctgcacgtttccgcgaaagataaaaacagcggtaaagagcagaagatcaccatcaaggcttcttctggtctgaacgaagatgaaatccagaaaatggtacgcgacgcagaagctaacgccgaagctgaccgtaagtttgaagagctggtacagactcgcaaccagggcgaccatctgctgcacagcacccgtaagcaggttgaagaagcaggcgacaaactgccggctgacgacaaaactgctatcgagtctgcgctgactgcactggaaactgctctgaaaggtgaagacaaagccgctatcgaagcgaaaatgcaggaactggcacaggtttcccagaaactgatggaaatcgcccagcagcaacatgcccagcagcagactgccggtgctgatgcttctgcaaacaacgcgaaagatgacgatgttgtcgacgctgaatttgaagaagtcaaagacaaaaaataatcgccctataaacgggtaattatactgacacgggcgaaggggaatttcctctccgcccgtgcattcatctaggggcaatttaaaaaagatggctaagcaagattattacgagattttaggcgtttccaaaacagcggaagagcgtgaaatcagaaaggcctacaaacgcctggccatgaaataccacccggaccgtaaccagggtgacaaagaggccgaggcgaaatttaaagagatcaaggaagcttatgaagttctgaccgactcgcaaaaacgtgcggcatacgatcagtatggtcatgctgcgtttgagcaaggtggcatgggcggcggcggttttggcggcggcgcagacttcagcgatatttttggtgacgttttcggcgatatttttggcggcggacgtggtcgtcaacgtgcggcgcgcggtgctgatttacgctataacatggagctcaccctcgaagaagctgtacgtggcgtgaccaaagagatccgcattccgactctggaagagtgtgacgtttgccacggtagcggtgcaaaaccaggtacacagccgcagacttgtccgacctgtcatggttctggtcaggtgcagatgcgccagggattcttcgctgtacagcagacctgtccacactgtcagggccgcggtacgctgatcaaagatccgtgcaacaaatgtcatggtcatggtcgtgttgagcgcagcaaaacgctgtccgttaaaatcccggcaggggtggacactggagaccgcatccgtcttgcgggcgaaggtgaagcgggcgagcatggcgcaccggcaggcgatctgtacgttcaggttcaggttaaacagcacccgattttcgagcgtgaaggcaacaacctgtattgcgaagtcccgatcaacttcgctatggcggcgctgggtggcgaaatcgaagtaccgacccttgatggtcgcgtcaaactgaaagtgcctggcgaaacccagaccggtaagctattccgtatgcgcggtaaaggcgtcaagtctgtccgcggtggcgcacagggtgatttgctgtgccgcgttgtcgtcgaaacaccggtaggcctgaacgaaaggcagaaacagctgctgcaagagctgcaagaaagcttcggtggcccaaccggcgagcacaacagcccgcgctcaaagagcttctttgatggtgtgaagaagttttttgacgacctgacccgctaacctgccggcctggttcaaccagtcggcagccgactagtggat

SEQ ID NO: 27 - DNA, 877 bp, synthetic construct
  source 1..877: mol_type = other DNA
atccatttaaatcacctggcagggcatgaagctgtttggcggggagcagcgcttcctcctggcggagtccggccacatcgccggcatcatcaacccgccggccgccaacaagtacggcttctggcacaacggggccgaggccgagagcccggagagctggctggcaggggcgacgcaccagggcggctcctggtggcccgagatgatgggctttatccagaaccgtgacgaagggtcagagcccgtccccgcgcgggtcccggaggaagggctggcccccgcccccggccactatgtcaaggtgcggctcaaccccgtgtttgcctgcccaacagaggaggacgccgcatgacgcttgcatgagtgccggcgtgcgtcatgcacagcgccggcaggcctgcaggttccctcccgtttccattgaaaggactacacacctgccggcctggttcaaccagtcggcagccggcgctggcgcccgcgtattgcggtgcagccagcgcggcgcacaaggcggcgggcgtttcgtttcgccgcccgtttcgcgggccgtcaaggcccgcgaatcgtttctgcccgcgcggcattcctcgctttttgcgccaattcaccgggttttccttaagccccgtcgcttttcttagtgccttgttgggcatagaatcagggcagcggcgcagccagcaccatgttcgtgcagcgcggccctcgcgggggcgaggctgcaggccgccacgcgcagccatgcgcgaacgggccaccagatggccggcacgacaacaagcagatggcgcgggcgataccgatttgcgcactgcaccccatgcggtgcagcagcgcgcaaacagcgatgacacaaggacagatttaaatccga

SEQ ID NO: 28 - DNA, 2836 bp, synthetic construct
  source 1..2836: mol_type = other DNA
atccatttaaatagcgcttcctcctggcggagtccggccacatcgccggcatcatcaacccgccggccgccaacaagtacggcttctggcacaacggggccgaggccgagagcccggagagctggctggcaggggcgacgcaccagggcggctcctggtggcccgagatgatgggctttatccagaaccgtgacgaagggtcagagcccgtccccgcgcgggtcccggaggaagggctggcccccgcccccggccactatgtcaaggtgcggctcaaccccgtgtttgcctgcccaacagaggaggacgccgcatgacgcttgcatgagtgccggcgtgcgtcatgcacagcgccggcaggcctgcaggttccctcccgtttccattgaaaggactacacaatgactgacgttgtgatcgtatcggccgcacgcaccgcggtaggcaaattcggcggctcgctggccaaggtgccggcccccgagctgggcgccatcgtcatcaaggccgcgctcgagcgcgccggcgtcaagccggagcaggtcagcgaagtaatcatgggccaggtgctgaccgccggctcgggacagaacccggcgcgccaggcggcgatcaaggccggactgccgcatatggttccggcgatgacgatcaacaaggtgtgcggttcgggcctgaaggccgtgatgctggccgccaatgcgatcgcctccggcgatgccgagatcgtcgtggctggcggccaggagaacatgagcgcggcgccgcacgtactgcccggctcgcgcgacggcttccgcatgggcgacgccaagctgatcgacacgatgatcgtcgacggcctgtgggacgtctataaccagtaccacatgggcatcaccgccgagaacgtggccaaggaatacggcatctcgcgcgaggcgcaggacgagttcgcggtcagctcgcagaacaaggccgaggccgcgcagaaggccgggcgcttcgacgaggaaatcgttccggtgatgatcccgcagcgcaagggcgaaccggtggcgttcgccaccgacgagttcgttcgccacggcgcgacgctcgagagcatcgccggcctgaagccggccttcgacaaggcgggcaccgtgaccgccgccaatgcctcgggcatcaacgatggcgccgccgccgtggtggtgatgtcggccgccaaggcgcgcgagctgggcctgaccccgcttgccacgatccgcgcctttgccaacgccggcgtcgacccgaaggtcatgggcatgggcccggtgccggcctcgcagcgctgcctgtcgcgcgccggctggagcgtgcaggacctggacctgatggagatcaacgaggcgttcgccgcgcaggcgctggcggtgcacaagcagatgggctgggacaccgacaaggtcaacgtcaatggcggcgcgatcgcgatcggccatccgatcggcgcgtcgggctgccgcattctggtgacgctgctgcacgaaatgaagcggcgcgatgcgaagaagggcctggcgtcgctgtgcatcggcggcggcatgggggtggcgctcgccgtggaacggtgaggaaggggttttccggggccgcgcgcggttggcgcggacccggcgacgataacgaagccaatcaaggagtggacatgactcagcgcattgcatacgtaacgggcggcatgggcggcatcggcaccgcgatctgccagcgcctggccaaggacggctttcgcgtgatcgcgggctgcggccccaactcgccgcgccgcgagcgctggctggaacagcagaaggcgctcggcttcgacttcattgcctccgagggcaacgtggccgactgggattcgaccaaggcggcgttcgacaaggtcaaggcggaggtcggcgaggtcgacgtgctgatcaacaatgcgggcatcacgcgcgacgtggtgttccgcaagatgacgcgcgccgactgggacgcggtgatcgacaccaacctgacctcgctgttcaacgtcaccaagcaggtgatcgacggcatggcggatcgcggctggggccggatcatcaatatctcgtcggtcaacgggcagaaggggcagttcggccagaccaactactcgaccgcgaaggccggcctgcacggcttcacgatggcgctggcgcaggaagtcgcgaccaagggcgtgacggtcaacacggtgtcgccgggctatatcgccaccgacatggtcaaggcgatccgtcaggacgtgctcgacaagatcgtcggcacgatccccgtcaagcgcctgggccagccggaggaaatcgcctcgatctgcgcctggctcgcgtcggaggaatccggcttcgccaccggtgccgacttctcgctgaacggcggcctgcacatgggctgacctgccggcctggttcaaccagtcggcagccggcgctggcgcccgcgtattgcggtgcagccagcgcggcgcacaaggcggcgggcgtttcgtttcgccgcccgtttcgcgggccgtcaaggcccgcgaatcgtttctgcccgcgcggcattcctcgctttttgcgccaattcaccgggttttccttaagccccgtcgcttttcttagtgccttgttgggcatagaatcagggcagcggcgcagccagcaccatgttcgtgcagcgcggccctcgcgggggcgaggctgcaggccgccacgcgcagccatgcgcgaacgggccaccagatggccggcacgacaacaagcagatggcgcgggcgataccgatttgcgcactgcaccccatgcggtgcagcagcgcgcaaacagcgatgacacaaggacagatttaaatccga